European Patent Application EP 4 360 643 A1, published May 1, 2024. Title: SOCS1 derived peptides for use in the treatment of liver diseases. Applicant: Universidad Autonoma de Madrid. The sequence listing filed with the application follows.

SEQUENCE LISTING (4 sequences)

SEQ ID NO: 1 - protein, 16 aa, synthetic construct
DTHFRTFRSHADYRRI

SEQ ID NO: 2 - protein, 10 aa, synthetic construct
  VARIANT 3: note = Cysteine at position 3 is substituted by acetaminomethyl-L-cysteine
DTCRQTFRSH

SEQ ID NO: 3 - protein, 10 aa, synthetic construct
  VARIANT 3: note = Cysteine at position 3 is substituted by acetaminomethyl-L-cysteine
DTCRQTFRKH

SEQ ID NO: 4 - protein, 10 aa, synthetic construct
  VARIANT 3: note = Cysteine at position 3 is substituted by acetaminomethyl-L-cysteine
  VARIANT 7: note = Phenylalanine is substituted by 1 naphthyl alanine
DTCRQTFRKH